European Patent Specification EP 3 697 808 B1, published January 3, 2024. Title: Neuroprotective Peptide. Applicant: University College Cardiff Consultants Limited. The sequence listing filed with the application follows.

SEQUENCE LISTING (19 sequences)

SEQ ID NO: 1 - protein, 32 aa, Homo sapiens
QGGGGGEPRRTEGVGPGVPGEVEMVKGQPFDV

SEQ ID NO: 2 - protein, 10 aa, Homo sapiens
GRKKRRQRRR

SEQ ID NO: 3 - protein, 16 aa, Homo sapiens
RQIKIWFQNRRMKWKK

SEQ ID NO: 4 - protein, 7 aa, Homo sapiens
RRRRRRR

SEQ ID NO: 5 - protein, 9 aa, Homo sapiens
  misc_feature (1)..(1): Xaa can be any naturally occurring amino acid
  misc_feature (9)..(9): Xaa can be any naturally occurring amino acid
XRRRRRRRX

SEQ ID NO: 6 - protein, 9 aa, Homo sapiens
  misc_feature (1)..(1): Xaa can be any naturally occurring amino acid
  misc_feature (5)..(5): Xaa can be any naturally occurring amino acid
XRRRXRRRR

SEQ ID NO: 7 - protein, 9 aa, Homo sapiens
  misc_feature (4)..(4): Xaa can be any naturally occurring amino acid
  misc_feature (9)..(9): Xaa can be any naturally occurring amino acid
RRRXRRRRX

SEQ ID NO: 8 - protein, 9 aa, Homo sapiens
  misc_feature (8)..(9): Xaa can be any naturally occurring amino acid
RRRRRRRXX

SEQ ID NO: 9 - protein, 9 aa, Homo sapiens
  misc_feature (1)..(2): Xaa can be any naturally occurring amino acid
XXRRRRRRR

SEQ ID NO: 10 - protein, 11 aa, Homo sapiens
RRRRRRRRRRR

SEQ ID NO: 11 - protein, 13 aa, Homo sapiens
  misc_feature (1)..(1): Xaa can be any naturally occurring amino acid
  misc_feature (7)..(7): Xaa can be any naturally occurring amino acid
XRRRRRXRRRRRR

SEQ ID NO: 12 - protein, 14 aa, Homo sapiens
  misc_feature (6)..(6): Xaa can be any naturally occurring amino acid
  misc_feature (14)..(14): Xaa can be any naturally occurring amino acid
RRRRRXRRRRRRRX

SEQ ID NO: 13 - protein, 22 aa, Homo sapiens
GAYDLRRRERQSRLRRRERQSR

SEQ ID NO: 14 - protein, 14 aa, Homo sapiens
SRRARRSPRHLGSG

SEQ ID NO: 15 - protein, 16 aa, Homo sapiens
LRRERQSRLRRERQSR

SEQ ID NO: 16 - protein, 19 aa, Homo sapiens
VKRGLKLRHVRPRVTRMDV

SEQ ID NO: 17 - protein, 16 aa, Homo sapiens
RKKRRRESRKKRRRES

SEQ ID NO: 18 - protein, 44 aa, Homo sapiens
GRKKRRQRRRPPQGGGGGEPRRTEGVGPGVPGEVEMVKGQPFDV

SEQ ID NO: 19 - protein, 43 aa, Homo sapiens
GRKKRRQRRRPPRVGPGVPEGVGVAVFGVKEPGQTGDVGPVGE